European Patent Specification EP 3 927 823 B1, published September 24, 2025. Title: A novel immuno-PCR method using cDNA display. Applicant: Epsilon Molecular Engineering Inc. The sequence listing filed with the application follows.

SEQUENCE LISTING (12 sequences)

SEQ ID NO: 1 - DNA, 367 bp, Artificial Sequence
  cDNA display molecule including full length of BDA
  misc_feature (1)..(367)
gatcccgcgaaattaatacgactcactataggggaagtatttttacaacaattaccaacaacaacaacaaacaacaacaacattacattttacattctacaactacaagccaccatggataacaaattcaacaaagaacaacaaaatgctttctatgaaatcttacatttacctaacttaaacgaagaacaacgcaatggtttcatccaaagcctaaaagatgacccaagccaaagcgctaaccttttagcagaagctaaaaagctaaatgatgctcaagcaccaaaagctgacaacaaattcaacgggggaggcagccatcatcatcatcatcacggcggaagcaggacggggggcggcgtggaaa

SEQ ID NO: 2 - DNA, 41 bp, Artificial Sequence
  Biotin-poly A-Inosine cnvK fragment (Biotin -poly A-Inosine cnvK fragment)
  misc_feature: y is inosine, k is cyanobinylcarbazole, and M is the amino-modifier C6 dT
aaaaaaaaaaaaaaaaaaaayttccakgccgccccccgmct

SEQ ID NO: 3 - DNA, 21 bp, Artificial Sequence
  BDA_pPCR(+)
  primer_bind (1)..(21)
ctacaagccaccatggataac

SEQ ID NO: 4 - DNA, 20 bp, Artificial Sequence
  BDA_pPCR(-)
  primer_bind (1)..(20)
gcttgggtcatcttttaggc

SEQ ID NO: 5 - DNA, 33 bp, Artificial Sequence
  Newleft
  primer_bind (1)..(33)
gatcccgcgaaattaatacgactcactataggg

SEQ ID NO: 6 - DNA, 22 bp, Artificial Sequence
  cnvK-NewYtag
  primer_bind (1)..(22)
tttccacgccgccccccgtcct

SEQ ID NO: 7 - DNA, 117 bp, Artificial Sequence
  T7 Omega
  exon (1)..(117)
gatcccgcgaaattaatacgactcactataggggaagtatttttacaacaattaccaacaacaacaacaaacaacaacaacattacattttacattctacaactacaagccaccatg

SEQ ID NO: 8 - DNA, 47 bp, Artificial Sequence
  1st Fw VHH
  primer_bind (1)..(47)
cattttacattctacaactacaagccaccatggcccaggtgcagctg

SEQ ID NO: 9 - DNA, 54 bp, Artificial Sequence
  1st Rv VHH
  primer_bind (1)..(54)
tttccacgccgccccccgtcctgcttccgccatgatgatgatgatgatgggaac

SEQ ID NO: 10 - DNA, 20 bp, Artificial Sequence
  GFP VHH qPCR FW
  primer_bind (1)..(20)
aacaccatcctgggcgatag

SEQ ID NO: 11 - DNA, 19 bp, Artificial Sequence
  GFP VHH qPCR Rv
  primer_bind (1)..(13)
gtgtttttggcgcgatcac

SEQ ID NO: 12 - DNA, 571 bp, Artificial Sequence
  cDNA display molecule including full length of anti-GFP VHH
  misc_feature (1)..(571)
gatcccgcgaaattaatacgactcactataggggaagtatttttacaacaattaccaacaacaacaacaaacaacaacaacattacattttacattctacaactacaagccaccatggcccaggtgcagctggttgaaagcggtggccgtctggtgcaggcgggtgatagcctgcgtctgagctgtgccgcaagcggtcgcacctttagcaccagcgccatggcatggtttcgtcaggccccgggccgtgaacgcgaatttgtggcggccattacctggaccgttggtaacaccatcctgggcgatagcgtgaaaggtcgttttaccattagccgtgatcgcgccaaaaacaccgtggatctgcagatggataatctggaaccggaagataccgcggtttattattgtagcgcccgtagccgcggttatgtgctgagcgttctgcgcagcgttgatagctatgattattggggtcagggcacccaggttacggtcagcggcggcggctcgggcggcggttcccatcatcatcatcatcatggcggaagcaggacggggggcggcgtggaaa